European Patent Application EP 4 431 110 A2, published September 18, 2024. Title: Enhanced receptor for improving immune cell function. Applicant: CHINEO MEDICAL TECHNOLOGY CO., LTD. The sequence listing filed with the application follows.

SEQUENCE LISTING (24 sequences)

SEQ ID NO: 1 - protein, 215 aa, synthetic construct
  REGION 1..215: note = PD1/CD28
MQIPQAPWPVVWAVLQLGWRPGWFLDSPDRPWNPPTFSPALLVVTEGDNATFTCSFSNTSESFVLNWYRMSPSNQTDKLAAFPEDRSQPGQDCRFRVTQLPNGRDFHMSVVRARRNDSGTYLCGAISLAPKAQIKESLRAELRVTERRAEVPTAHCPSPLFPGPSKPFWVLVVVGGVLACYSLLVTVAFIIFWVRSKRSRLLHSDYMNMTPRRPG

SEQ ID NO: 2 - protein, 220 aa, synthetic construct
  REGION 1..220: note = PD1/ 41BBz
MQIPQAPWPVVWAVLQLGWRPGWFLDSPDRPWNPPTFSPALLVVTEGDNATFTCSFSNTSESFVLNWYRMSPSNQTDKLAAFPEDRSQPGQDCRFRVTQLPNGRDFHMSVVRARRNDSGTYLCGAISLAPKAQIKESLRAELRVTERRAEVPTAHFLALTSTALLFLLFFLTLRFSVVKRGRKKLLYIFKQPFMRPVQTTQEEDGCSCRFPEEEEGGCEL

SEQ ID NO: 3 - protein, 213 aa, synthetic construct
  REGION 1..213: note = PD1/ICOS
MQIPQAPWPVVWAVLQLGWRPGWFLDSPDRPWNPPTFSPALLVVTEGDNATFTCSFSNTSESFVLNWYRMSPSNQTDKLAAFPEDRSQPGQDCRFRVTQLPNGRDFHMSVVRARRNDSGTYLCGAISLAPKAQIKESLRAELRVTERRAEVPTAHWLPIGCAAFVVVCILGCILICWLTKKKYSSSVHDPNGEYMFMRAVNTAKKSRLTDVTL

SEQ ID NO: 4 - protein, 300 aa, synthetic construct
  REGION 1..300: note = PDL1/ CD28
DIQMTQSPSSLSASVGDRVTITCRASQDVSTAVAWYQQKPGKAPKLLIYSASFLYSGVPSRFSGSGSGTDFTLTISSLQPEDFATYYCQQYLYHPATFGQGTKVEIKGGGGSGGGGSGGGGSEVQLVESGGGLVQPGGSLRLSCAASGFTFSDSWIHWVRQAPGKGLEWVAWISPYGGSTYYADSVKGRFTISADTSKNTAYLQMNSLRAEDTAVYYCARRHWPGGFDYWGQGTLVTVSSCPSPLFPGPSKPFWVLVVVGGVLACYSLLVTVAFIIFWVRSKRSRLLHSDYMNMTPRRPG

SEQ ID NO: 5 - protein, 305 aa, synthetic construct
  REGION 1..305: note = PDL1/ 41BBz
DIQMTQSPSSLSASVGDRVTITCRASQDVSTAVAWYQQKPGKAPKLLIYSASFLYSGVPSRFSGSGSGTDFTLTISSLQPEDFATYYCQQYLYHPATFGQGTKVEIKGGGGSGGGGSGGGGSEVQLVESGGGLVQPGGSLRLSCAASGFTFSDSWIHWVRQAPGKGLEWVAWISPYGGSTYYADSVKGRFTISADTSKNTAYLQMNSLRAEDTAVYYCARRHWPGGFDYWGQGTLVTVSSFLALTSTALLFLLFFLTLRFSVVKRGRKKLLYIFKQPFMRPVQTTQEEDGCSCRFPEEEEGGCEL

SEQ ID NO: 6 - protein, 298 aa, synthetic construct
  REGION 1..298: note = PDL1/ICOS
DIQMTQSPSSLSASVGDRVTITCRASQDVSTAVAWYQQKPGKAPKLLIYSASFLYSGVPSRFSGSGSGTDFTLTISSLQPEDFATYYCQQYLYHPATFGQGTKVEIKGGGGSGGGGSGGGGSEVQLVESGGGLVQPGGSLRLSCAASGFTFSDSWIHWVRQAPGKGLEWVAWISPYGGSTYYADSVKGRFTISADTSKNTAYLQMNSLRAEDTAVYYCARRHWPGGFDYWGQGTLVTVSSWLPIGCAAFVVVCILGCILICWLTKKKYSSSVHDPNGEYMFMRAVNTAKKSRLTDVTL

SEQ ID NO: 7 - protein, 441 aa, synthetic construct
  REGION 1..441: note = K4D5-628/CD28
DFQVQIFSFLLISASVIMSRGDIQMTQSPSSLSASVGDRVTITCRASQDVNTAVAWYQQKPGKAPKLLIYSASFLYSGVPSRFSGSRSGTDFTLTISSLQPEDFATYYCQQHYTTPPTFGQGTKVEIKRTGSTSGSGKPGSGEGSEVQLVESGGGLVQPGGSLRLSCAASGFNIKDTYIHWVRQAPGKGLEWVARIYPTNGYTRYADSVKGRFTISADTSKNTAYLQMNSLRAEDTAVYYCSRWGGDGFYAMDVWGQGTLVTVSSAAATTTPAPRPPTPAPTIASQPLSLRPEACRPAAGGAVHTRGLDFACDFWVLVVVGGVLACYSLLVTVAFIIFWVRSKRSRLLHSDYMNMTPRRPGPTRKHYQPYAPPRDFAAYRSCPSPLFPGPSKPFWVLVVVGGVLACYSLLVTVAFIIFWVRSKRSRLLHSDYMNMTPRRPG

SEQ ID NO: 8 - protein, 441 aa, synthetic construct
  REGION 1..441: note = K4D5-728/CD28
DFQVQIFSFLLISASVIMSRGDIQMTQSPSSLSASVGDRVTITCRASQDVNTAVAWYQQKPGKAPKLLIYSASFLESGVPSRFSGSRSGTDFTLTISSLQPEDFATYYCQQHYTTPPTFGQGTKVEIKRTGSTSGSGKPGSGEGSEVQLVESGGGLVQPGGSLRLSCAASGFNIKDTYIHWVRQAPGKGLEWVARIYPTNGYTRYADSVKGRFTISADTSKNTAYLQMNSLRAEDTAVYYCSRWGGDGFYAMDVWGQGTLVTVSSAAATTTPAPRPPTPAPTIASQPLSLRPEACRPAAGGAVHTRGLDFACDFWVLVVVGGVLACYSLLVTVAFIIFWVRSKRSRLLHSDYMNMTPRRPGPTRKHYQPYAPPRDFAAYRSCPSPLFPGPSKPFWVLVVVGGVLACYSLLVTVAFIIFWVRSKRSRLLHSDYMNMTPRRPG

SEQ ID NO: 9 - protein, 441 aa, synthetic construct
  REGION 1..441: note = K4D5728/CD28
DFQVQIFSFLLISASVIMSRGDIQMTQSPSSLSASVGDRVTITCRASQDVNTAVAWYQQKPGKAPKLLIYSASFLYSGVPSRFSGSRSGTDFTLTISSLQPEDFATYYCQQHYTTPPTFGQGTKVEIKRTGSTSGSGKPGSGEGSEVQLVESGGGLVQPGGSLRLSCAASGFNIKDTYIHWVRQAPGKGLEWVARIYPTNGYTRYADSVKGRFTISADTSKNTAYLQMNSLRAEDTAVYYCSRWGGDGFVAMDVWGQGTLVTVSSAAATTTPAPRPPTPAPTIASQPLSLRPEACRPAAGGAVHTRGLDFACDFWVLVVVGGVLACYSLLVTVAFIIFWVRSKRSRLLHSDYMNMTPRRPGPTRKHYQPYAPPRDFAAYRSCPSPLFPGPSKPFWVLVVVGGVLACYSLLVTVAFIIFWVRSKRSRLLHSDYMNMTPRRPG

SEQ ID NO: 10 - protein, 446 aa, synthetic construct
  REGION 1..446: note = K4D5-628/41BBz
DFQVQIFSFLLISASVIMSRGDIQMTQSPSSLSASVGDRVTITCRASQDVNTAVAWYQQKPGKAPKLLIYSASFLYSGVPSRFSGSRSGTDFTLTISSLQPEDFATYYCQQHYTTPPTFGQGTKVEIKRTGSTSGSGKPGSGEGSEVQLVESGGGLVQPGGSLRLSCAASGFNIKDTYIHWVRQAPGKGLEWVARIYPTNGYTRYADSVKGRFTISADTSKNTAYLQMNSLRAEDTAVYYCSRWGGDGFYAMDVWGQGTLVTVSSAAATTTPAPRPPTPAPTIASQPLSLRPEACRPAAGGAVHTRGLDFACDFWVLVVVGGVLACYSLLVTVAFIIFWVRSKRSRLLHSDYMNMTPRRPGPTRKHYQPYAPPRDFAAYRSFLALTSTALLFLLFFLTLRFSVVKRGRKKLLYIFKQPFMRPVQTTQEEDGCSCRFPEEEEGGCEL

SEQ ID NO: 11 - protein, 446 aa, synthetic construct
  REGION 1..446: note = K4D5-728/41BBz
DFQVQIFSFLLISASVIMSRGDIQMTQSPSSLSASVGDRVTITCRASQDVNTAVAWYQQKPGKAPKLLIYSASFLESGVPSRFSGSRSGTDFTLTISSLQPEDFATYYCQQHYTTPPTFGQGTKVEIKRTGSTSGSGKPGSGEGSEVQLVESGGGLVQPGGSLRLSCAASGFNIKDTYIHWVRQAPGKGLEWVARIYPTNGYTRYADSVKGRFTISADTSKNTAYLQMNSLRAEDTAVYYCSRWGGDGFYAMDVWGQGTLVTVSSAAATTTPAPRPPTPAPTIASQPLSLRPEACRPAAGGAVHTRGLDFACDFWVLVVVGGVLACYSLLVTVAFIIFWVRSKRSRLLHSDYMNMTPRRPGPTRKHYQPYAPPRDFAAYRSFLALTSTALLFLLFFLTLRFSVVKRGRKKLLYIFKQPFMRPVQTTQEEDGCSCRFPEEEEGGCEL

SEQ ID NO: 12 - protein, 446 aa, synthetic construct
  REGION 1..446: note = K4D5728/41BBz
DFQVQIFSFLLISASVIMSRGDIQMTQSPSSLSASVGDRVTITCRASQDVNTAVAWYQQKPGKAPKLLIYSASFLYSGVPSRFSGSRSGTDFTLTISSLQPEDFATYYCQQHYTTPPTFGQGTKVEIKRTGSTSGSGKPGSGEGSEVQLVESGGGLVQPGGSLRLSCAASGFNIKDTYIHWVRQAPGKGLEWVARIYPTNGYTRYADSVKGRFTISADTSKNTAYLQMNSLRAEDTAVYYCSRWGGDGFVAMDVWGQGTLVTVSSAAATTTPAPRPPTPAPTIASQPLSLRPEACRPAAGGAVHTRGLDFACDFWVLVVVGGVLACYSLLVTVAFIIFWVRSKRSRLLHSDYMNMTPRRPGPTRKHYQPYAPPRDFAAYRSFLALTSTALLFLLFFLTLRFSVVKRGRKKLLYIFKQPFMRPVQTTQEEDGCSCRFPEEEEGGCEL

SEQ ID NO: 13 - protein, 439 aa, synthetic construct
  REGION 1..439: note = K4D5-628/ICOS
DFQVQIFSFLLISASVIMSRGDIQMTQSPSSLSASVGDRVTITCRASQDVNTAVAWYQQKPGKAPKLLIYSASFLYSGVPSRFSGSRSGTDFTLTISSLQPEDFATYYCQQHYTTPPTFGQGTKVEIKRTGSTSGSGKPGSGEGSEVQLVESGGGLVQPGGSLRLSCAASGFNIKDTYIHWVRQAPGKGLEWVARIYPTNGYTRYADSVKGRFTISADTSKNTAYLQMNSLRAEDTAVYYCSRWGGDGFYAMDVWGQGTLVTVSSAAATTTPAPRPPTPAPTIASQPLSLRPEACRPAAGGAVHTRGLDFACDFWVLVVVGGVLACYSLLVTVAFIIFWVRSKRSRLLHSDYMNMTPRRPGPTRKHYQPYAPPRDFAAYRSWLPIGCAAFVVVCILGCILICWLTKKKYSSSVHDPNGEYMFMRAVNTAKKSRLTDVTL

SEQ ID NO: 14 - protein, 439 aa, synthetic construct
  REGION 1..439: note = K4D5-728/ICOSz
DFQVQIFSFLLISASVIMSRGDIQMTQSPSSLSASVGDRVTITCRASQDVNTAVAWYQQKPGKAPKLLIYSASFLESGVPSRFSGSRSGTDFTLTISSLQPEDFATYYCQQHYTTPPTFGQGTKVEIKRTGSTSGSGKPGSGEGSEVQLVESGGGLVQPGGSLRLSCAASGFNIKDTYIHWVRQAPGKGLEWVARIYPTNGYTRYADSVKGRFTISADTSKNTAYLQMNSLRAEDTAVYYCSRWGGDGFYAMDVWGQGTLVTVSSAAATTTPAPRPPTPAPTIASQPLSLRPEACRPAAGGAVHTRGLDFACDFWVLVVVGGVLACYSLLVTVAFIIFWVRSKRSRLLHSDYMNMTPRRPGPTRKHYQPYAPPRDFAAYRSWLPIGCAAFVVVCILGCILICWLTKKKYSSSVHDPNGEYMFMRAVNTAKKSRLTDVTL

SEQ ID NO: 15 - protein, 439 aa, synthetic construct
  REGION 1..439: note = K4D5728/ICOS
DFQVQIFSFLLISASVIMSRGDIQMTQSPSSLSASVGDRVTITCRASQDVNTAVAWYQQKPGKAPKLLIYSASFLYSGVPSRFSGSRSGTDFTLTISSLQPEDFATYYCQQHYTTPPTFGQGTKVEIKRTGSTSGSGKPGSGEGSEVQLVESGGGLVQPGGSLRLSCAASGFNIKDTYIHWVRQAPGKGLEWVARIYPTNGYTRYADSVKGRFTISADTSKNTAYLQMNSLRAEDTAVYYCSRWGGDGFVAMDVWGQGTLVTVSSAAATTTPAPRPPTPAPTIASQPLSLRPEACRPAAGGAVHTRGLDFACDFWVLVVVGGVLACYSLLVTVAFIIFWVRSKRSRLLHSDYMNMTPRRPGPTRKHYQPYAPPRDFAAYRSWLPIGCAAFVVVCILGCILICWLTKKKYSSSVHDPNGEYMFMRAVNTAKKSRLTDVTL

SEQ ID NO: 16 - protein, 111 aa, synthetic construct
  REGION 1..111: note = NKG2D/CD28
MGWIRGRRSRHSWEMSEFHNYNLDLKKSDFSTRWQKQRCPVVKSKCRENASCPSPLFPGPSKPFWVLVVVGGVLACYSLLVTVAFIIFWVRSKRSRLLHSDYMNMTPRRPG

SEQ ID NO: 17 - protein, 116 aa, synthetic construct
  REGION 1..116: note = NKG2D/41BBz
MGWIRGRRSRHSWEMSEFHNYNLDLKKSDFSTRWQKQRCPVVKSKCRENASFLALTSTALLFLLFFLTLRFSVVKRGRKKLLYIFKQPFMRPVQTTQEEDGCSCRFPEEEEGGCEL

SEQ ID NO: 18 - protein, 109 aa, synthetic construct
  REGION 1..109: note = NKG2D/ICOS
MGWIRGRRSRHSWEMSEFHNYNLDLKKSDFSTRWQKQRCPVVKSKCRENASWLPIGCAAFVVVCILGCILICWLTKKKYSSSVHDPNGEYMFMRAVNTAKKSRLTDVTL

SEQ ID NO: 19 - protein, 304 aa, synthetic construct
  REGION 1..304: note = CD47 mAb/CD28
DIVMTQSPLSLPVTPGEPASISCRSSQSIVYSNGNTYLGWYLQKPGQSPQLLIYKVSNRFSGVPDRFSGSGSGTDFTLKISRVEAEDVGVYYCFQGSHVPYTFGQGTKLEIKGGGGSGGGGSGGGGSQVQLVQSGAEVKKPGASVKVSCKASGYTFTNYNMHWVRQAPGQRLEWMGTIYPGNDDTSYNQKFKDRVTITADTSASTAYMELSSLRSEDTAVYYCARGGYRAMDYWGQGTLVTVSSCPSPLFPGPSKPFWVLVVVGGVLACYSLLVTVAFIIFWVRSKRSRLLHSDYMNMTPRRPG

SEQ ID NO: 20 - protein, 309 aa, synthetic construct
  REGION 1..309: note = CD47 mAb/41BBz
DIVMTQSPLSLPVTPGEPASISCRSSQSIVYSNGNTYLGWYLQKPGQSPQLLIYKVSNRFSGVPDRFSGSGSGTDFTLKISRVEAEDVGVYYCFQGSHVPYTFGQGTKLEIKGGGGSGGGGSGGGGSQVQLVQSGAEVKKPGASVKVSCKASGYTFTNYNMHWVRQAPGQRLEWMGTIYPGNDDTSYNQKFKDRVTITADTSASTAYMELSSLRSEDTAVYYCARGGYRAMDYWGQGTLVTVSSFLALTSTALLFLLFFLTLRFSVVKRGRKKLLYIFKQPFMRPVQTTQEEDGCSCRFPEEEEGGCEL

SEQ ID NO: 21 - protein, 302 aa, synthetic construct
  REGION 1..302: note = CD47 mAb/ICOS
DIVMTQSPLSLPVTPGEPASISCRSSQSIVYSNGNTYLGWYLQKPGQSPQLLIYKVSNRFSGVPDRFSGSGSGTDFTLKISRVEAEDVGVYYCFQGSHVPYTFGQGTKLEIKGGGGSGGGGSGGGGSQVQLVQSGAEVKKPGASVKVSCKASGYTFTNYNMHWVRQAPGQRLEWMGTIYPGNDDTSYNQKFKDRVTITADTSASTAYMELSSLRSEDTAVYYCARGGYRAMDYWGQGTLVTVSSWLPIGCAAFVVVCILGCILICWLTKKKYSSSVHDPNGEYMFMRAVNTAKKSRLTDVTL

SEQ ID NO: 22 - protein, 430 aa, synthetic construct
  REGION 1..430: note = SIRP / CD28
MEPAGPAPGRLGPLLCLLLAASCAWSGVAGEEELQVIQPDKSVSVAAGESAILHCTVTSLIPVGPIQWFRGAGPARELIYNQKEGHFPRVTTVSESTKRENMDFSISISNITPADAGTYYCVKFRKGSPDTEFKSGAGTELSVRAKPSAPVVSGPAARATPQHTVSFTCESHGFSPRDITLKWFKNGNELSDFQTNVDPVGESVSYSIHSTAKVVLTREDVHSQVICEVAHVTLQGDPLRGTANLSETIRVPPTLEVTQQPVRAENQVNVTCQVRKFYPQRLQLTWLENGNVSRTETASTVTENKDGTYNWMSWLLVNVSAHRDDVKLTCQVEHDGQPAVSKSHDLKVSAHPKEQGSNTAAENTGSNERNCPSPLFPGPSKPFWVLVVVGGVLACYSLLVTVAFIIFWVRSKRSRLLHSDYMNMTPRRPG

SEQ ID NO: 23 - protein, 435 aa, synthetic construct
  REGION 1..435: note = SIRP /41BBz
MEPAGPAPGRLGPLLCLLLAASCAWSGVAGEEELQVIQPDKSVSVAAGESAILHCTVTSLIPVGPIQWFRGAGPARELIYNQKEGHFPRVTTVSESTKRENMDFSISISNITPADAGTYYCVKFRKGSPDTEFKSGAGTELSVRAKPSAPVVSGPAARATPQHTVSFTCESHGFSPRDITLKWFKNGNELSDFQTNVDPVGESVSYSIHSTAKVVLTREDVHSQVICEVAHVTLQGDPLRGTANLSETIRVPPTLEVTQQPVRAENQVNVTCQVRKFYPQRLQLTWLENGNVSRTETASTVTENKDGTYNWMSWLLVNVSAHRDDVKLTCQVEHDGQPAVSKSHDLKVSAHPKEQGSNTAAENTGSNERNFLALTSTALLFLLFFLTLRFSVVKRGRKKLLYIFKQPFMRPVQTTQEEDGCSCRFPEEEEGGCEL

SEQ ID NO: 24 - protein, 428 aa, synthetic construct
  REGION 1..428: note = SIRP /ICOS
MEPAGPAPGRLGPLLCLLLAASCAWSGVAGEEELQVIQPDKSVSVAAGESAILHCTVTSLIPVGPIQWFRGAGPARELIYNQKEGHFPRVTTVSESTKRENMDFSISISNITPADAGTYYCVKFRKGSPDTEFKSGAGTELSVRAKPSAPVVSGPAARATPQHTVSFTCESHGFSPRDITLKWFKNGNELSDFQTNVDPVGESVSYSIHSTAKVVLTREDVHSQVICEVAHVTLQGDPLRGTANLSETIRVPPTLEVTQQPVRAENQVNVTCQVRKFYPQRLQLTWLENGNVSRTETASTVTENKDGTYNWMSWLLVNVSAHRDDVKLTCQVEHDGQPAVSKSHDLKVSAHPKEQGSNTAAENTGSNERNWLPIGCAAFVVVCILGCILICWLTKKKYSSSVHDPNGEYMFMRAVNTAKKSRLTDVTL